European Patent Specification EP 3 366 702 B1, published August 9, 2023. Title: ANTI-IL-17 ANTIBODIES. Applicant: Eli Lilly and Company. The sequence listing filed with the application follows.

SEQUENCE LISTING (280 sequences)

SEQ ID NO: 1 - protein, 155 aa, Homo sapiens
MTPGKTSLVSLLLLLSLEAIVKAGITIPRNPGCPNSEDKNFPRTVMVNLNIHNRNTNTNPKRSSDYYNRSTSPWNLHRNEDPERYPSVIWEAKCRHLGCINADGNVDYHMNSVPIQQEILVLRREPPHCPNSFRLEKILVSVGCTCVTPIVHHVA

SEQ ID NO: 2 - protein, 178 aa, Homo sapiens
MDWPHNLLFLLTISIFLGLGPWPKWKRKGQGRPGPLAPGPHQVPLDLVSRMKPYARMEEYERNIEEMVAQLRNSSELAQRKCEVNLQLWMSNKRSLSPWGYSINHDPSRIPVDLPEARCLCLGCVNPFTMWEDRSMVSVPVFSQVPVRRRLCPPPPRTGPCRQRAVMETIAVGCTCIF

SEQ ID NO: 3 - protein, 196 aa, Homo sapiens
MTLLPGLLFLTWLHTCLAHHDPSLRGHPHSHGTPHCYSAEELPLQAPPHLIARGAKWGQALPVALVSSLEAASHRGRHERPSATTQCPVLRPEEVLEADTHQRSISPWRYRVDTDEDRYPQKLAFAECLCRGCIDARTGRETAALNSVRLLQSLLVLRRRPCSRDGSGLPTPGAFAFHTEFIHVPVGCTCVLPRSV

SEQ ID NO: 4 - protein, 202 aa, Homo sapiens
MLVAGFLLALPPSWAAGAPRAGRRPARPRGCADRPEELLEQLYGRLAAGVLSAFHHTLQLGPREQARNASCPAGGRPADRRFRPPTNLRSVSPWAYRISYDPARYPRYLPEAYCLCRGCLTGLFGEEDVRFRSAPVYMPTVVLRRTPACAGGRSVYTEAYVTIPVGCTCVPEPEKDADSINSSIDKQGAKLLLGPNDAPAGP

SEQ ID NO: 5 - protein, 177 aa, Homo sapiens
MRERPRLGEDSSLISLFLQVVAFLAMVMGTHTYSHWPSCCPSKGQDTSEELLRWSTVPVPPLEPARPNRHPESCRASEDGPLNSRAISPWRYELDRDLNRLPQDLYHARCLCPHCVSLQTGSHMDPRGNSELLYHNQTVFYRRPCHGEKGTHKGYCLEFFLYRVSLACVCVRPRVMG

SEQ ID NO: 6 - protein, 132 aa, Homo sapiens
MVKYLLLSILGLAFLSEAAARKIPKVGHTFFQKPESCSMSRNIESRSTSPWNYTVTWDPNRYPSEVVQAQCRNLGCINAQGKEDISMNSVPIQQETLVVRRKHQGCSVSFQLEKVLVTVGCTCVTPVIHHVQ

SEQ ID NO: 7 - protein, 158 aa, Mus sp.
MSPGRASSVSLMLLLLLSLAATVKAAAIIPQSSACPNTEAKDFLQNVKVNLKVFNSLGAKVSSRRPSDYLNRSTSPWTLHRNEDPDRYPSVIWEAQCRHQRCVNAEGKLDHHMNSVLIQQEILVLKREPESCPFTFRVEKMLVGVGCTCVASIVRQAA

SEQ ID NO: 8 - protein, 158 aa, Rattus rattus
MSPRRIPSMCLMLLLLLNLEATVKAAVLIPQSSVCPNAEANNFLQNVKVNLKVINSLSSKASSRRPSDYLNRSTSPWTLSRNEDPDRYPSVIWEAQCRHQRCVNAEGKLDHHMNSVLIQQEILVLKREPEKCPFTFRVEKMLVGVGCTCVSSIVRHAS

SEQ ID NO: 9 - protein, 153 aa, Oryctolagus cuniculus
MSLGRISSVSLLLLLCLVATVKNGIAMPRNPGCPNAEDKNFPQNVKVSLNILNKSVNSRRPSDYYNRSTSPWTLHRNEDRERYPSVIWEAKCRHLGCVNAEGNEDHHMNSVPIQQEILVLRRESQHCPHSFRLEKMLVAVGCTCVTPIIHHMA

SEQ ID NO: 10 - protein, 155 aa, Macaca fascicularis
MTPGKTSLVLLLLLLSLEAIVKAGIAIPRNSGCPNSEDKNFPRTVMVNLNIHNRNTSTNPKRSSDYYNRSTSPWNLHRNEDPERYPSVIWEAKCRHLGCVKADGNVDYHMNSVPIQQEILVLRREPRHCPNSFRLEKILVSVGCTCVTPIVHHVA

SEQ ID NO: 11 - protein, 10 aa, Artificial
  Synthetic construct
GYSFTDYNMN

SEQ ID NO: 12 - protein, 10 aa, Artificial
  Synthetic construct
GYSFTDYNIN

SEQ ID NO: 13 - protein, 10 aa, Artificial
  Synthetic construct
GYSFTDYNLN

SEQ ID NO: 14 - protein, 10 aa, Artificial
  Synthetic construct
GYSFGDYNMN

SEQ ID NO: 15 - protein, 10 aa, Artificial
  Synthetic construct
GYSFRDYNMN

SEQ ID NO: 16 - protein, 10 aa, Artificial
  Synthetic construct
GYSFTWYNMN

SEQ ID NO: 17 - protein, 10 aa, Artificial
  Synthetic construct
GYSFNDYNMN

SEQ ID NO: 18 - protein, 10 aa, Artificial
  Synthetic construct
GYSFTDYNMS

SEQ ID NO: 19 - protein, 10 aa, Artificial
  Synthetic construct
GYSFTDYNTN

SEQ ID NO: 20 - protein, 10 aa, Artificial
  Synthetic construct
GYSFPDYNMN

SEQ ID NO: 21 - protein, 10 aa, Artificial
  Synthetic construct
HYSFTDYNMN

SEQ ID NO: 22 - protein, 10 aa, Artificial
  Synthetic construct
GYHFTDYNMN

SEQ ID NO: 23 - protein, 10 aa, Artificial
  Synthetic construct
GYPFTDYNMN

SEQ ID NO: 24 - protein, 10 aa, Artificial
  Synthetic construct
GYSFTDFNMN

SEQ ID NO: 25 - protein, 10 aa, Artificial
  Synthetic construct
GYSFTDYHLG

SEQ ID NO: 26 - protein, 10 aa, Artificial
  Synthetic construct
GYSFTDYHIH

SEQ ID NO: 27 - protein, 10 aa, Artificial
  Synthetic construct
GYSFTDYHMS

SEQ ID NO: 28 - protein, 10 aa, Artificial
  Synthetic construct
GYSFTDYHIS

SEQ ID NO: 29 - protein, 17 aa, Artificial
  Synthetic construct
VINPNYGTTDYNQRFKG

SEQ ID NO: 30 - protein, 17 aa, Artificial
  Synthetic construct
VINPMYGTTDYNQRFKG

SEQ ID NO: 31 - protein, 17 aa, Artificial
  Synthetic construct
VINPAYGTTDYNQRFKG

SEQ ID NO: 32 - protein, 17 aa, Artificial
  Synthetic construct
VINPEYGTTDYNQRFKG

SEQ ID NO: 33 - protein, 10 aa, Artificial
  Synthetic construct
YDYATGTGAY

SEQ ID NO: 34 - protein, 10 aa, Artificial
  Synthetic construct
YDYWTGTGGY

SEQ ID NO: 35 - protein, 10 aa, Artificial
  Synthetic construct
YDYWTGTGAY

SEQ ID NO: 36 - protein, 10 aa, Artificial
  Synthetic construct
YDYATGTGLY

SEQ ID NO: 37 - protein, 10 aa, Artificial
  Synthetic construct
YDYATGTGGY

SEQ ID NO: 38 - protein, 10 aa, Artificial
  Synthetic construct
YDYATGTGVY

SEQ ID NO: 39 - protein, 10 aa, Artificial
  Synthetic construct
YDYHTGTGGY

SEQ ID NO: 40 - protein, 10 aa, Artificial
  Synthetic construct
YDYATGTGTY

SEQ ID NO: 41 - protein, 10 aa, Artificial
  Synthetic construct
YDYFTGTGGY

SEQ ID NO: 42 - protein, 10 aa, Artificial
  Synthetic construct
YDYFTGTGPY

SEQ ID NO: 43 - protein, 10 aa, Artificial
  Synthetic construct
YDYYTGTGGY

SEQ ID NO: 44 - protein, 10 aa, Artificial
  Synthetic construct
YDYSTGTGGY

SEQ ID NO: 45 - protein, 10 aa, Artificial
  Synthetic construct
YDYSTGTGAY

SEQ ID NO: 46 - protein, 10 aa, Artificial
  Synthetic construct
YDAFTGTGAY

SEQ ID NO: 47 - protein, 10 aa, Artificial
  Synthetic construct
YDYYTGTGAY

SEQ ID NO: 48 - protein, 10 aa, Artificial
  Synthetic construct
YDYHTGTGAY

SEQ ID NO: 49 - protein, 10 aa, Artificial
  Synthetic construct
YDYLTGTGAY

SEQ ID NO: 50 - protein, 10 aa, Artificial
  Synthetic construct
YDYATSTGAY

SEQ ID NO: 51 - protein, 10 aa, Artificial
  Synthetic construct
YDYAPGTGAY

SEQ ID NO: 52 - protein, 10 aa, Artificial
  Synthetic construct
YDYFTGTGVY

SEQ ID NO: 53 - protein, 10 aa, Artificial
  Synthetic construct
YDYYTGTGVY

SEQ ID NO: 54 - protein, 10 aa, Artificial
  Synthetic construct
YDPATGTGAY

SEQ ID NO: 55 - protein, 10 aa, Artificial
  Synthetic construct
YDYHTGTGVY

SEQ ID NO: 56 - protein, 119 aa, Artificial
  Synthetic construct
QVQLVQSGAEVKKPGSSVKVSCKASGYSFTDYNMNWVRQAPGQGLEWMGVINPNYGTTDYNQRFKGRVTITADESTSTAYMELSSLRSEDTAVYYCARYDYATGTGAYWGQGTLVTVSS

SEQ ID NO: 57 - protein, 119 aa, Artificial
  Synthetic construct
QVQLVQSGAEVKKPGSSVKVSCKASGYSFTDYNMNWVRQAPGQGLEWMGVINPNYGTTDYNQRFKGRVTITADESTSTAYMELSSLRSEDTAVYYCARYDYWTGTGGYWGQGTLVTVSS

SEQ ID NO: 58 - protein, 119 aa, Artificial
  Synthetic construct
QVQLVQSGAEVKKPGSSVKVSCKASGYSFTDYNMNWVRQAPGQGLEWMGVINPNYGTTDYNQRFKGRVTITADESTSTAYMELSSLRSEDTAVYYCARYDYWTGTGAYWGQGTLVTVSS

SEQ ID NO: 59 - protein, 119 aa, Artificial
  Synthetic construct
QVQLVQSGAEVKKPGSSVKVSCKASGYSFTDYNMNWVRQAPGQGLEWMGVINPNYGTTDYNQRFKGRVTITADESTSTAYMELSSLRSEDTAVYYCARYDYATGTGLYWGQGTLVTVSS

SEQ ID NO: 60 - protein, 119 aa, Artificial
  Synthetic construct
QVQLVQSGAEVKKPGSSVKVSCKASGYSFTDYNMNWVRQAPGQGLEWMGVINPNYGTTDYNQRFKGRVTITADESTSTAYMELSSLRSEDTAVYYCARYDYATGTGGYWGQGTLVTVSS

SEQ ID NO: 61 - protein, 119 aa, Artificial
  Synthetic construct
QVQLVQSGAEVKKPGSSVKVSCKASGYSFTDYNMNWVRQAPGQGLEWMGVINPNYGTTDYNQRFKGRVTITADESTSTAYMELSSLRSEDTAVYYCARYDYATGTGVYWGQGTLVTVSS

SEQ ID NO: 62 - protein, 119 aa, Artificial
  Synthetic construct
QVQLVQSGAEVKKPGSSVKVSCKASGYSFTDYNMNWVRQAPGQGLEWMGVINPNYGTTDYNQRFKGRVTITADESTSTAYMELSSLRSEDTAVYYCARYDYHTGTGGYWGQGTLVTVSS

SEQ ID NO: 63 - protein, 119 aa, Artificial
  Synthetic construct
QVQLVQSGAEVKKPGSSVKVSCKASGYSFTDYNMNWVRQAPGQGLEWMGVINPNYGTTDYNQRFKGRVTITADESTSTAYMELSSLRSEDTAVYYCARYDYATGTGTYWGQGTLVTVSS

SEQ ID NO: 64 - protein, 119 aa, Artificial
  Synthetic construct
QVQLVQSGAEVKKPGSSVKVSCKASGYSFTDYNMNWVRQAPGQGLEWMGVINPNYGTTDYNQRFKGRVTITADESTSTAYMELSSLRSEDTAVYYCARYDYFTGTGGYWGQGTLVTVSS

SEQ ID NO: 65 - protein, 119 aa, Artificial
  Synthetic construct
QVQLVQSGAEVKKPGSSVKVSCKASGYSFTDYNMNWVRQAPGQGLEWMGVINPNYGTTDYNQRFKGRVTITADESTSTAYMELSSLRSEDTAVYYCARYDYFTGTGPYWGQGTLVTVSS

SEQ ID NO: 66 - protein, 119 aa, Artificial
  Synthetic construct
QVQLVQSGAEVKKPGSSVKVSCKASGYSFTDYNMNWVRQAPGQGLEWMGVINPNYGTTDYNQRFKGRVTITADESTSTAYMELSSLRSEDTAVYYCARYDYYTGTGGYWGQGTLVTVSS

SEQ ID NO: 67 - protein, 119 aa, Artificial
  Synthetic construct
QVQLVQSGAEVKKPGSSVKVSCKASGYSFTDYNMNWVRQAPGQGLEWMGVINPNYGTTDYNQRFKGRVTITADESTSTAYMELSSLRSEDTAVYYCARYDYSTGTGGYWGQGTLVTVSS

SEQ ID NO: 68 - protein, 119 aa, Artificial
  Synthetic construct
QVQLVQSGAEVKKPGSSVKVSCKASGYSFTDYNINWVRQAPGQGLEWMGVINPNYGTTDYNQRFKGRVTITADESTSTAYMELSSLRSEDTAVYYCARYDYATGTGAYWGQGTLVTVSS

SEQ ID NO: 69 - protein, 119 aa, Artificial
  Synthetic construct
QVQLVQSGAEVKKPGSSVKVSCKASGYSFTDYNLNWVRQAPGQGLEWMGVINPNYGTTDYNQRFKGRVTITADESTSTAYMELSSLRSEDTAVYYCARYDYATGTGAYWGQGTLVTVSS

SEQ ID NO: 70 - protein, 119 aa, Artificial
  Synthetic construct
QVQLVQSGAEVKKPGSSVKVSCKASGYSFGDYNMNWVRQAPGQGLEWMGVINPNYGTTDYNQRFKGRVTITADESTSTAYMELSSLRSEDTAVYYCARYDYATGTGAYWGQGTLVTVSS

SEQ ID NO: 71 - protein, 119 aa, Artificial
  Synthetic construct
QVQLVQSGAEVKKPGSSVKVSCKASGYSFRDYNMNWVRQAPGQGLEWMGVINPNYGTTDYNQRFKGRVTITADESTSTAYMELSSLRSEDTAVYYCARYDYATGTGAYWGQGTLVTVSS

SEQ ID NO: 72 - protein, 119 aa, Artificial
  Synthetic construct
QVQLVQSGAEVKKPGSSVKVSCKASGYSFTWYNMNWVRQAPGQGLEWMGVINPNYGTTDYNQRFKGRVTITADESTSTAYMELSSLRSEDTAVYYCARYDYATGTGAYWGQGTLVTVSS

SEQ ID NO: 73 - protein, 119 aa, Artificial
  Synthetic construct
QVQLVQSGAEVKKPGSSVKVSCKASGYSFNDYNMNWVRQAPGQGLEWMGVINPNYGTTDYNQRFKGRVTITADESTSTAYMELSSLRSEDTAVYYCARYDYATGTGAYWGQGTLVTVSS

SEQ ID NO: 74 - protein, 119 aa, Artificial
  Synthetic construct
QVQLVQSGAEVKKPGSSVKVSCKASGYSFTDYNMSWVRQAPGQGLEWMGVINPNYGTTDYNQRFKGRVTITADESTSTAYMELSSLRSEDTAVYYCARYDYATGTGAYWGQGTLVTVSS

SEQ ID NO: 75 - protein, 119 aa, Artificial
  Synthetic construct
QVQLVQSGAEVKKPGSSVKVSCKASGYSFTDYNTNWVRQAPGQGLEWMGVINPNYGTTDYNQRFKGRVTITADESTSTAYMELSSLRSEDTAVYYCARYDYATGTGAYWGQGTLVTVSS

SEQ ID NO: 76 - protein, 119 aa, Artificial
  Synthetic construct
QVQLVQSGAEVKKPGSSVKVSCKASGYSFPDYNMNWVRQAPGQGLEWMGVINPNYGTTDYNQRFKGRVTITADESTSTAYMELSSLRSEDTAVYYCARYDYATGTGAYWGQGTLVTVSS

SEQ ID NO: 77 - protein, 119 aa, Artificial
  Synthetic construct
QVQLVQSGAEVKKPGSSVKVSCKASHYSFTDYNMNWVRQAPGQGLEWMGVINPNYGTTDYNQRFKGRVTITADESTSTAYMELSSLRSEDTAVYYCARYDYATGTGAYWGQGTLVTVSS

SEQ ID NO: 78 - protein, 119 aa, Artificial
  Synthetic construct
QVQLVQSGAEVKKPGSSVKVSCKASGYHFTDYNMNWVRQAPGQGLEWMGVINPNYGTTDYNQRFKGRVTITADESTSTAYMELSSLRSEDTAVYYCARYDYATGTGAYWGQGTLVTVSS

SEQ ID NO: 79 - protein, 119 aa, Artificial
  Synthetic construct
QVQLVQSGAEVKKPGSSVKVSCKASGYPFTDYNMNWVRQAPGQGLEWMGVINPNYGTTDYNQRFKGRVTITADESTSTAYMELSSLRSEDTAVYYCARYDYATGTGAYWGQGTLVTVSS

SEQ ID NO: 80 - protein, 119 aa, Artificial
  Synthetic construct
QVQLVQSGAEVKKPGSSVKVSCKASGYSFTDFNMNWVRQAPGQGLEWMGVINPNYGTTDYNQRFKGRVTITADESTSTAYMELSSLRSEDTAVYYCARYDYATGTGAYWGQGTLVTVSS

SEQ ID NO: 81 - protein, 119 aa, Artificial
  Synthetic construct
QVQLVQSGAEVKKPGSSVKVSCKASGYSFTDYNMNWVRQAPGQGLEWMGVINPMYGTTDYNQRFKGRVTITADESTSTAYMELSSLRSEDTAVYYCARYDYATGTGAYWGQGTLVTVSS

SEQ ID NO: 82 - protein, 119 aa, Artificial
  Synthetic construct
QVQLVQSGAEVKKPGSSVKVSCKASGYSFTDYNMNWVRQAPGQGLEWMGVINPAYGTTDYNQRFKGRVTITADESTSTAYMELSSLRSEDTAVYYCARYDYATGTGAYWGQGTLVTVSS

SEQ ID NO: 83 - protein, 119 aa, Artificial
  Synthetic construct
QVQLVQSGAEVKKPGSSVKVSCKASGYSFTDYNMNWVRQAPGQGLEWMGVINPEYGTTDYNQRFKGRVTITADESTSTAYMELSSLRSEDTAVYYCARYDYATGTGAYWGQGTLVTVSS

SEQ ID NO: 84 - protein, 119 aa, Artificial
  Synthetic construct
QVQLVQSGAEVKKPGSSVKVSCKASGYSFTDYNMNWVRQAPGQGLEWMGVINPNYGTTDYNQRFKGRVTITADESTSTAYMELSSLRSEDTAVYYCARYDYSTGTGAYWGQGTLVTVSS

SEQ ID NO: 85 - protein, 119 aa, Artificial
  Synthetic construct
QVQLVQSGAEVKKPGSSVKVSCKASGYSFTDYNMNWVRQAPGQGLEWMGVINPNYGTTDYNQRFKGRVTITADESTSTAYMELSSLRSEDTAVYYCARYDYFTGTGAYWGQGTLVTVSS

SEQ ID NO: 86 - protein, 119 aa, Artificial
  Synthetic construct
QVQLVQSGAEVKKPGSSVKVSCKASGYSFTDYNMNWVRQAPGQGLEWMGVINPNYGTTDYNQRFKGRVTITADESTSTAYMELSSLRSEDTAVYYCARYDYYTGTGAYWGQGTLVTVSS

SEQ ID NO: 87 - protein, 119 aa, Artificial
  Synthetic construct
QVQLVQSGAEVKKPGSSVKVSCKASGYSFTDYNMNWVRQAPGQGLEWMGVINPNYGTTDYNQRFKGRVTITADESTSTAYMELSSLRSEDTAVYYCARYDYHTGTGAYWGQGTLVTVSS

SEQ ID NO: 88 - protein, 119 aa, Artificial
  Synthetic construct
QVQLVQSGAEVKKPGSSVKVSCKASGYSFTDYNMNWVRQAPGQGLEWMGVINPNYGTTDYNQRFKGRVTITADESTSTAYMELSSLRSEDTAVYYCARYDYLTGTGAYWGQGTLVTVSS

SEQ ID NO: 89 - protein, 119 aa, Artificial
  Synthetic construct
QVQLVQSGAEVKKPGSSVKVSCKASGYSFTDYNMNWVRQAPGQGLEWMGVINPNYGTTDYNQRFKGRVTITADESTSTAYMELSSLRSEDTAVYYCARYDYATSTGAYWGQGTLVTVSS

SEQ ID NO: 90 - protein, 119 aa, Artificial
  Synthetic construct
QVQLVQSGAEVKKPGSSVKVSCKASGYSFTDYNMNWVRQAPGQGLEWMGVINPNYGTTDYNQRFKGRVTITADESTSTAYMELSSLRSEDTAVYYCARYDYAPGTGAYWGQGTLVTVSS

SEQ ID NO: 91 - protein, 119 aa, Artificial
  Synthetic construct
QVQLVQSGAEVKKPGSSVKVSCKASGYSFTDYNMNWVRQAPGQGLEWMGVINPNYGTTDYNQRFKGRVTITADESTSTAYMELSSLRSEDTAVYYCARYDYFTGTGVYWGQGTLVTVSS

SEQ ID NO: 92 - protein, 119 aa, Artificial
  Synthetic construct
QVQLVQSGAEVKKPGSSVKVSCKASGYSFTDYNMNWVRQAPGQGLEWMGVINPNYGTTDYNQRFKGRVTITADESTSTAYMELSSLRSEDTAVYYCARYDYYTGTGVYWGQGTLVTVSS

SEQ ID NO: 93 - protein, 119 aa, Artificial
  Synthetic construct
QVQLVQSGAEVKKPGSSVKVSCKASGYSFTDYNMNWVRQAPGQGLEWMGVINPNYGTTDYNQRFKGRVTITADESTSTAYMELSSLRSEDTAVYYCARYDPATGTGAYWGQGTLVTVSS

SEQ ID NO: 94 - protein, 119 aa, Artificial
  Synthetic construct
QVQLVQSGAEVKKPGSSVKVSCKASGYSFTDYHLGWVRQAPGQGLEWMGVINPNYGTTDYNQRFKGRVTITADESTSTAYMELSSLRSEDTAVYYCARYDYFTGTGAYWGQGTLVTVSS

SEQ ID NO: 95 - protein, 119 aa, Artificial
  Synthetic construct
QVQLVQSGAEVKKPGSSVKVSCKASGYSFTDYHIHWVRQAPGQGLEWMGVINPNYGTTDYNQRFKGRVTITADESTSTAYMELSSLRSEDTAVYYCARYDYFTGTGAYWGQGTLVTVSS

SEQ ID NO: 96 - protein, 119 aa, Artificial
  Synthetic construct
QVQLVQSGAEVKKPGSSVKVSCKASGYSFTDYHIHWVRQAPGQGLEWMGVINPNYGTTDYNQRFKGRVTITADESTSTAYMELSSLRSEDTAVYYCARYDYHTGTGVYWGQGTLVTVSS

SEQ ID NO: 97 - protein, 119 aa, Artificial
  Synthetic construct
QVQLVQSGAEVKKPGSSVKVSCKASGYSFTDYHIHWVRQAPGQGLEWMGVINPNYGTTDYNQRFKGRVTITADESTSTAYMELSSLRSEDTAVYYCARYDYHTGTGAYWGQGTLVTVSS

SEQ ID NO: 98 - protein, 119 aa, Artificial
  Synthetic construct
QVQLVQSGAEVKKPGSSVKVSCKASGYSFTDYHIHWVRQAPGQGLEWMGVINPNYGTTDYNQRFKGRVTITADESTSTAYMELSSLRSEDTAVYYCARYDYYTGTGAYWGQGTLVTVSS

SEQ ID NO: 99 - protein, 119 aa, Artificial
  Synthetic construct
QVQLVQSGAEVKKPGSSVKVSCKASGYSFTDYHMSWVRQAPGQGLEWMGVINPNYGTTDYNQRFKGRVTITADESTSTAYMELSSLRSEDTAVYYCARYDYFTGTGAYWGQGTLVTVSS

SEQ ID NO: 100 - protein, 119 aa, Artificial
  Synthetic construct
QVQLVQSGAEVKKPGSSVKVSCKASGYSFTDYHIHWVRQAPGQGLEWMGVINPNYGTTDYNQRFKGRVTITADESTSTAYMELSSLRSEDTAVYYCARYDYFTGTGVYWGQGTLVTVSS

SEQ ID NO: 101 - protein, 119 aa, Artificial
  Synthetic construct
QVQLVQSGAEVKKPGSSVKVSCKASGYSFTDYHMSWVRQAPGQGLEWMGVINPNYGTTDYNQRFKGRVTITADESTSTAYMELSSLRSEDTAVYYCARYDYHTGTGAYWGQGTLVTVSS

SEQ ID NO: 102 - protein, 119 aa, Artificial
  Synthetic construct
QVQLVQSGAEVKKPGSSVKVSCKASGYSFTDYHIHWVRQAPGQGLEWMGVINPEYGTTDYNQRFKGRVTITADESTSTAYMELSSLRSEDTAVYYCARYDYFTGTGAYWGQGTLVTVSS

SEQ ID NO: 103 - protein, 119 aa, Artificial
  Synthetic construct
QVQLVQSGAEVKKPGSSVKVSCKASGYSFTDYHIHWVRQAPGQGLEWMGVINPEYGTTDYNQRFKGRVTITADESTSTAYMELSSLRSEDTAVYYCARYDYATGTGAYWGQGTLVTVSS

SEQ ID NO: 104 - protein, 119 aa, Artificial; identical to SEQ ID NO: 102
  Synthetic construct

SEQ ID NO: 105 - protein, 119 aa, Artificial
  Synthetic construct
QVQLVQSGAEVKKPGSSVKVSCKASGYSFTDYHIHWVRQAPGQGLEWMGVINPEYGTTDYNQRFKGRVTITADESTSTAYMELSSLRSEDTAVYYCARYDYYTGTGAYWGQGTLVTVSS

SEQ ID NO: 106 - protein, 119 aa, Artificial; identical to SEQ ID NO: 98
  Synthetic construct

SEQ ID NO: 107 - protein, 119 aa, Artificial
  Synthetic construct
QVQLVQSGAEVKKPGSSVKVSCKASGYSFTDYHLGWVRQAPGQGLEWMGVINPEYGTTDYNQRFKGRVTITADESTSTAYMELSSLRSEDTAVYYCARYDYHTGTGAYWGQGTLVTVSS

SEQ ID NO: 108 - protein, 119 aa, Artificial; identical to SEQ ID NO: 98
  Synthetic construct

SEQ ID NO: 109 - protein, 119 aa, Artificial
  Synthetic construct
QVQLVQSGAEVKKPGSSVKVSCKASGYSFTDYHMSWVRQAPGQGLEWMGVINPEYGTTDYNQRFKGRVTITADESTSTAYMELSSLRSEDTAVYYCARYDYFTGTGAYWGQGTLVTVSS

SEQ ID NO: 110 - protein, 119 aa, Artificial
  Synthetic construct
QVQLVQSGAEVKKPGSSVKVSCKASGYSFTDYHMSWVRQAPGQGLEWMGVINPNYGTTDYNQRFKGRVTITADESTSTAYMELSSLRSEDTAVYYCARYDYYTGTGAYWGQGTLVTVSS

SEQ ID NO: 111 - protein, 119 aa, Artificial
  Synthetic construct
QVQLVQSGAEVKKPGSSVKVSCKASGYSFTDYHISWVRQAPGQGLEWMGVINPEYGTTDYNQRFKGRVTITADESTSTAYMELSSLRSEDTAVYYCARYDYYTGTGVYWGQGTLVTVSS

SEQ ID NO: 112 - protein, 119 aa, Artificial
  Synthetic construct
QVQLVQSGAEVKKPGSSVKVSCKASGYSFTDYHISWVRQAPGQGLEWMGVINPMYGTTDYNQRFKGRVTITADESTSTAYMELSSLRSEDTAVYYCARYDYYTGTGVYWGQGTLVTVSS

SEQ ID NO: 113 - protein, 119 aa, Artificial
  Synthetic construct
QVQLVQSGAEVKKPGSSVKVSCKASGYSFTDYHISWVRQAPGQGLEWMGVINPEYGTTDYNQRFKGRVTITADESTSTAYMELSSLRSEDTAVYYCARYDYFTGTGAYWGQGTLVTVSS

SEQ ID NO: 114 - protein, 119 aa, Artificial
  Synthetic construct
QVQLVQSGAEVKKPGSSVKVSCKASGYSFTDYHIHWVRQAPGQGLEWMGVINPMYGTTDYNQRFKGRVTITADESTSTAYMELSSLRSEDTAVYYCARYDYYTGTGVYWGQGTLVTVSS

SEQ ID NO: 115 - protein, 119 aa, Artificial
  Synthetic construct
QVQLVQSGAEVKKPGSSVKVSCKASGYSFTDYHIHWVRQAPGQGLEWMGVINPNYGTTDYNQRFKGRVTITADESTSTAYMELSSLRSEDTAVYYCARYDYYTGTGVYWGQGTLVTVSS

SEQ ID NO: 116 - protein, 119 aa, Artificial
  Synthetic construct
QVQLVQSGAEVKKPGSSVKVSCKASGYSFTDYNMNWVRQAPGQGLEWMGVINPMYGTTDYNQRFKGRVTITADESTSTAYMELSSLRSEDTAVYYCARYDYYTGTGVYWGQGTLVTVSS

SEQ ID NO: 117 - protein, 119 aa, Artificial
  Synthetic construct
QVQLVQSGAEVKKPGSSVKVSCKASGYSFTDYHIHWVRQAPGQGLEWMGVINPEYGTTDYNQRFKGRVTITADESTSTAYMELSSLRSEDTAVYYCARYDYFTGTGVYWGQGTLVTVSS

SEQ ID NO: 118 - protein, 119 aa, Artificial
  Synthetic construct
QVQLVQSGAEVKKPGSSVKVSCKASGYSFTDYHIHWVRQAPGQGLEWMGVINPMYGTTDYNQRFKGRVTITADESTSTAYMELSSLRSEDTAVYYCARYDYFTGTGVYWGQGTLVTVSS

SEQ ID NO: 119 - protein, 119 aa, Artificial
  Synthetic construct
QVQLVQSGAEVKKPGSSVKVSCKASGYSFTDYHMSWVRQAPGQGLEWMGVINPMYGTTDYNQRFKGRVTITADESTSTAYMELSSLRSEDTAVYYCARYDYYTGTGAYWGQGTLVTVSS

SEQ ID NO: 120 - protein, 119 aa, Artificial; identical to SEQ ID NO: 118
  Synthetic construct

SEQ ID NO: 121 - protein, 119 aa, Artificial
  Synthetic construct
QVQLVQSGAEVKKPGSSVKVSCKASGYSFTDYHMSWVRQAPGQGLEWMGVINPMYGTTDYNQRFKGRVTITADESTSTAYMELSSLRSEDTAVYYCARYDYFTGTGVYWGQGTLVTVSS

SEQ ID NO: 122 - protein, 16 aa, Artificial
  Synthetic construct
RSSQSLVHSRGNTYLH

SEQ ID NO: 123 - protein, 16 aa, Artificial
  Synthetic construct
RSSQSLVHSHGNTYLH

SEQ ID NO: 124 - protein, 16 aa, Artificial
  Synthetic construct
RSSQSLVHSNGNTYLH

SEQ ID NO: 125 - protein, 16 aa, Artificial
  Synthetic construct
RSSQSLVHSYGNTYLH

SEQ ID NO: 126 - protein, 16 aa, Artificial
  Synthetic construct
RSSQSVVHSRGNTYLH

SEQ ID NO: 127 - protein, 16 aa, Artificial
  Synthetic construct
VSSQSLVHSRGNTYLH

SEQ ID NO: 128 - protein, 16 aa, Artificial
  Synthetic construct
RSSASLVHSRGNTYLH

SEQ ID NO: 129 - protein, 16 aa, Artificial
  Synthetic construct
RSSQSLKHSRGNTYLH

SEQ ID NO: 130 - protein, 16 aa, Artificial
  Synthetic construct
RSSQSLRHSRGNTYLH

SEQ ID NO: 131 - protein, 16 aa, Artificial
  Synthetic construct
RSSRSLVHSRGNTYLH

SEQ ID NO: 132 - protein, 16 aa, Artificial
  Synthetic construct
RSHQSLVHSRGNTYLH

SEQ ID NO: 133 - protein, 16 aa, Artificial
  Synthetic construct
RSSQSLVHSRGNTFLH

SEQ ID NO: 134 - protein, 16 aa, Artificial
  Synthetic construct
RSSQSLVHNRGNTYLH

SEQ ID NO: 135 - protein, 16 aa, Artificial
  Synthetic construct
RSSQSLVHSRGRTYLH

SEQ ID NO: 136 - protein, 16 aa, Artificial
  Synthetic construct
RSSQSLVHRRGNTYLH

SEQ ID NO: 137 - protein, 16 aa, Artificial
  Synthetic construct
RSSQSLVHSRGNTYTH

SEQ ID NO: 138 - protein, 16 aa, Artificial
  Synthetic construct
RSSQSLVHSRGNTYSH

SEQ ID NO: 139 - protein, 16 aa, Artificial
  Synthetic construct
RSSQSLVHSRGNTYHH

SEQ ID NO: 140 - protein, 16 aa, Artificial
  Synthetic construct
RSSQSLVHARGNTYLH

SEQ ID NO: 141 - protein, 16 aa, Artificial
  Synthetic construct
RSSQSLVHSRGNTWLH

SEQ ID NO: 142 - protein, 16 aa, Artificial
  Synthetic construct
RSSQSLVHSRGNVYLH

SEQ ID NO: 143 - protein, 16 aa, Artificial
  Synthetic construct
RSSQSLVHSRGKTYLH

SEQ ID NO: 144 - protein, 16 aa, Artificial
  Synthetic construct
RSSQSLVHLRGNTYLH

SEQ ID NO: 145 - protein, 16 aa, Artificial
  Synthetic construct
RSSKSLVHSRGNTFLH

SEQ ID NO: 146 - protein, 16 aa, Artificial
  Synthetic construct
RSSQSLRHSRGNTFLH

SEQ ID NO: 147 - protein, 16 aa, Artificial
  Synthetic construct
RSSQSLKHSRGNTFLH

SEQ ID NO: 148 - protein, 16 aa, Artificial
  Synthetic construct
RSSRSLVHSRGNTFLH

SEQ ID NO: 149 - protein, 16 aa, Artificial
  Synthetic construct
RSSQSLKHSHGNTYLH

SEQ ID NO: 150 - protein, 7 aa, Artificial
  Synthetic construct
KVSNRFS

SEQ ID NO: 151 - protein, 7 aa, Artificial
  Synthetic construct
IVSNRFS

SEQ ID NO: 152 - protein, 7 aa, Artificial
  Synthetic construct
KVSNRFH

SEQ ID NO: 153 - protein, 7 aa, Artificial
  Synthetic construct
KVANRFS

SEQ ID NO: 154 - protein, 7 aa, Artificial
  Synthetic construct
KVSVRFS

SEQ ID NO: 155 - protein, 7 aa, Artificial
  Synthetic construct
KVSNNFS

SEQ ID NO: 156 - protein, 7 aa, Artificial
  Synthetic construct
KVDNRFS

SEQ ID NO: 157 - protein, 7 aa, Artificial
  Synthetic construct
KVTNRFS

SEQ ID NO: 158 - protein, 7 aa, Artificial
  Synthetic construct
KVSNIFS

SEQ ID NO: 159 - protein, 7 aa, Artificial
  Synthetic construct
KVSTRFS

SEQ ID NO: 160 - protein, 7 aa, Artificial
  Synthetic construct
KVRNRFS

SEQ ID NO: 161 - protein, 7 aa, Artificial
  Synthetic construct
KVPNRFS

SEQ ID NO: 162 - protein, 7 aa, Artificial
  Synthetic construct
KVSNRFV

SEQ ID NO: 163 - protein, 7 aa, Artificial
  Synthetic construct
KVSNRIS

SEQ ID NO: 164 - protein, 7 aa, Artificial
  Synthetic construct
KVSNRFT

SEQ ID NO: 165 - protein, 7 aa, Artificial
  Synthetic construct
KVSNRNS

SEQ ID NO: 166 - protein, 7 aa, Artificial
  Synthetic construct
KVHNRFS

SEQ ID NO: 167 - protein, 7 aa, Artificial
  Synthetic construct
KVSNRFI

SEQ ID NO: 168 - protein, 9 aa, Artificial
  Synthetic construct
SQSTHLPFT

SEQ ID NO: 169 - protein, 9 aa, Artificial
  Synthetic construct
SQSTHYPFT

SEQ ID NO: 170 - protein, 9 aa, Artificial
  Synthetic construct
SQSTHIPFT

SEQ ID NO: 171 - protein, 9 aa, Artificial
  Synthetic construct
SQSLHVPFT

SEQ ID NO: 172 - protein, 9 aa, Artificial
  Synthetic construct
SQSTHEPFT

SEQ ID NO: 173 - protein, 9 aa, Artificial
  Synthetic construct
NQSTHVPFT

SEQ ID NO: 174 - protein, 9 aa, Artificial
  Synthetic construct
SQTTHVPFT

SEQ ID NO: 175 - protein, 9 aa, Artificial
  Synthetic construct
SQSMHVPFT

SEQ ID NO: 176 - protein, 9 aa, Artificial
  Synthetic construct
SQTTHLPFT

SEQ ID NO: 177 - protein, 9 aa, Artificial
  Synthetic construct
SQSTSLPFT

SEQ ID NO: 178 - protein, 112 aa, Artificial
  Synthetic construct
DIVMTQTPLSLSVTPGQPASISCRSSQSLVHSRGNTYLHWYLQKPGQSPQLLIYKVSNRFSGVPDRFSGSGSGTDFTLKISRVEAEDVGVYYCSQSTHLPFTFGQGTKLEIK

SEQ ID NO: 179 - protein, 112 aa, Artificial
  Synthetic construct
DIVMTQTPLSLSVTPGQPASISCRSSQSLVHSRGNTYLHWYLQKPGQSPQLLIYKVSNRFSGVPDRFSGSGSGTDFTLKISRVEAEDVGVYYCSQSTHYPFTFGQGTKLEIK

SEQ ID NO: 180 - protein, 112 aa, Artificial
  Synthetic construct
DIVMTQTPLSLSVTPGQPASISCRSSQSLVHSHGNTYLHWYLQKPGQSPQLLIYKVSNRFSGVPDRFSGSGSGTDFTLKISRVEAEDVGVYYCSQSTHLPFTFGQGTKLEIK

SEQ ID NO: 181 - protein, 112 aa, Artificial
  Synthetic construct
DIVMTQTPLSLSVTPGQPASISCRSSQSLVHSNGNTYLHWYLQKPGQSPQLLIYKVSNRFSGVPDRFSGSGSGTDFTLKISRVEAEDVGVYYCSQSTHLPFTFGQGTKLEIK

SEQ ID NO: 182 - protein, 112 aa, Artificial
  Synthetic construct
DIVMTQTPLSLSVTPGQPASISCRSSQSLVHSNGNTYLHWYLQKPGQSPQLLIYKVSNRFSGVPDRFSGSGSGTDFTLKISRVEAEDVGVYYCSQSTHYPFTFGQGTKLEIK

SEQ ID NO: 183 - protein, 112 aa, Artificial
  Synthetic construct
DIVMTQTPLSLSVTPGQPASISCRSSQSLVHSYGNTYLHWYLQKPGQSPQLLIYKVSNRFSGVPDRFSGSGSGTDFTLKISRVEAEDVGVYYCSQSTHYPFTFGQGTKLEIK

SEQ ID NO: 184 - protein, 112 aa, Artificial; identical to SEQ ID NO: 182
  Synthetic construct

SEQ ID NO: 185 - protein, 112 aa, Artificial; identical to SEQ ID NO: 182
  Synthetic construct

SEQ ID NO: 186 - protein, 112 aa, Artificial; identical to SEQ ID NO: 182
  Synthetic construct

SEQ ID NO: 187 - protein, 112 aa, Artificial
  Synthetic construct
DIVMTQTPLSLSVTPGQPASISCRSSQSLVHSHGNTYLHWYLQKPGQSPQLLIYKVSNRFSGVPDRFSGSGSGTDFTLKISRVEAEDVGVYYCSQSTHYPFTFGQGTKLEIK

SEQ ID NO: 188 - protein, 112 aa, Artificial; identical to SEQ ID NO: 187
  Synthetic construct

SEQ ID NO: 189 - protein, 112 aa, Artificial; identical to SEQ ID NO: 182
  Synthetic construct

SEQ ID NO: 190 - protein, 112 aa, Artificial; identical to SEQ ID NO: 182
  Synthetic construct

SEQ ID NO: 191 - protein, 112 aa, Artificial
  Synthetic construct
DIVMTQTPLSLSVTPGQPASISCRSSKSLVHSRGNTYLHWYLQKPGQSPQLLIYKVSNRFSGVPDRFSGSGSGTDFTLKISRVEAEDVGVYYCSQSTHYPFTFGQGTKLEIK

SEQ ID NO: 192 - protein, 112 aa, Artificial
  Synthetic construct
DIVMTQTPLSLSVTPGQPASISCRSSQSVVHSRGNTYLHWYLQKPGQSPQLLIYKVSNRFSGVPDRFSGSGSGTDFTLKISRVEAEDVGVYYCSQSTHYPFTFGQGTKLEIK

SEQ ID NO: 193 - protein, 112 aa, Artificial
  Synthetic construct
DIVMTQTPLSLSVTPGQPASISCVSSQSLVHSRGNTYLHWYLQKPGQSPQLLIYKVSNRFSGVPDRFSGSGSGTDFTLKISRVEAEDVGVYYCSQSTHYPFTFGQGTKLEIK

SEQ ID NO: 194 - protein, 112 aa, Artificial
  Synthetic construct
DIVMTQTPLSLSVTPGQPASISCRSSASLVHSRGNTYLHWYLQKPGQSPQLLIYKVSNRFSGVPDRFSGSGSGTDFTLKISRVEAEDVGVYYCSQSTHYPFTFGQGTKLEIK

SEQ ID NO: 195 - protein, 112 aa, Artificial
  Synthetic construct
DIVMTQTPLSLSVTPGQPASISCRSSQSLKHSRGNTYLHWYLQKPGQSPQLLIYKVSNRFSGVPDRFSGSGSGTDFTLKISRVEAEDVGVYYCSQSTHYPFTFGQGTKLEIK

SEQ ID NO: 196 - protein, 112 aa, Artificial
  Synthetic construct
DIVMTQTPLSLSVTPGQPASISCRSSQSLRHSRGNTYLHWYLQKPGQSPQLLIYKVSNRFSGVPDRFSGSGSGTDFTLKISRVEAEDVGVYYCSQSTHYPFTFGQGTKLEIK

SEQ ID NO: 197 - protein, 112 aa, Artificial
  Synthetic construct
DIVMTQTPLSLSVTPGQPASISCRSSRSLVHSRGNTYLHWYLQKPGQSPQLLIYKVSNRFSGVPDRFSGSGSGTDFTLKISRVEAEDVGVYYCSQSTHYPFTFGQGTKLEIK

SEQ ID NO: 198 - protein, 112 aa, Artificial
  Synthetic construct
DIVMTQTPLSLSVTPGQPASISCRSHQSLVHSRGNTYLHWYLQKPGQSPQLLIYKVSNRFSGVPDRFSGSGSGTDFTLKISRVEAEDVGVYYCSQSTHYPFTFGQGTKLEIK

SEQ ID NO: 199 - protein, 112 aa, Artificial
  Synthetic construct
DIVMTQTPLSLSVTPGQPASISCRSSQSLVHSRGNTFLHWYLQKPGQSPQLLIYKVSNRFSGVPDRFSGSGSGTDFTLKISRVEAEDVGVYYCSQSTHYPFTFGQGTKLEIK

SEQ ID NO: 200 - protein, 112 aa, Artificial
  Synthetic construct
DIVMTQTPLSLSVTPGQPASISCRSSQSLVHNRGNTYLHWYLQKPGQSPQLLIYKVSNRFSGVPDRFSGSGSGTDFTLKISRVEAEDVGVYYCSQSTHYPFTFGQGTKLEIK

SEQ ID NO: 201 - protein, 112 aa, Artificial
  Synthetic construct
DIVMTQTPLSLSVTPGQPASISCRSSQSLVHSRGRTYLHWYLQKPGQSPQLLIYKVSNRFSGVPDRFSGSGSGTDFTLKISRVEAEDVGVYYCSQSTHYPFTFGQGTKLEIK

SEQ ID NO: 202 - protein, 112 aa, Artificial
  Synthetic construct
DIVMTQTPLSLSVTPGQPASISCRSSQSLVHRRGNTYLHWYLQKPGQSPQLLIYKVSNRFSGVPDRFSGSGSGTDFTLKISRVEAEDVGVYYCSQSTHYPFTFGQGTKLEIK

SEQ ID NO: 203 - protein, 112 aa, Artificial
  Synthetic construct
DIVMTQTPLSLSVTPGQPASISCRSSQSLVHSRGNTYTHWYLQKPGQSPQLLIYKVSNRFSGVPDRFSGSGSGTDFTLKISRVEAEDVGVYYCSQSTHYPFTFGQGTKLEIK

SEQ ID NO: 204 - protein, 112 aa, Artificial
  Synthetic construct
DIVMTQTPLSLSVTPGQPASISCRSSQSLVHSRGNTYSHWYLQKPGQSPQLLIYKVSNRFSGVPDRFSGSGSGTDFTLKISRVEAEDVGVYYCSQSTHYPFTFGQGTKLEIK

SEQ ID NO: 205 - protein, 112 aa, Artificial
  Synthetic construct
DIVMTQTPLSLSVTPGQPASISCRSSQSLVHSRGNTYHHWYLQKPGQSPQLLIYKVSNRFSGVPDRFSGSGSGTDFTLKISRVEAEDVGVYYCSQSTHYPFTFGQGTKLEIK

SEQ ID NO: 206 - protein, 112 aa, Artificial
  Synthetic construct
DIVMTQTPLSLSVTPGQPASISCRSSQSLVHARGNTYLHWYLQKPGQSPQLLIYKVSNRFSGVPDRFSGSGSGTDFTLKISRVEAEDVGVYYCSQSTHYPFTFGQGTKLEIK

SEQ ID NO: 207 - protein, 112 aa, Artificial
  Synthetic construct
DIVMTQTPLSLSVTPGQPASISCRSSQSLVHSRGNTWLHWYLQKPGQSPQLLIYKVSNRFSGVPDRFSGSGSGTDFTLKISRVEAEDVGVYYCSQSTHYPFTFGQGTKLEIK

SEQ ID NO: 208 - protein, 112 aa, Artificial
  Synthetic construct
DIVMTQTPLSLSVTPGQPASISCRSSQSLVHSRGNVYLHWYLQKPGQSPQLLIYKVSNRFSGVPDRFSGSGSGTDFTLKISRVEAEDVGVYYCSQSTHYPFTFGQGTKLEIK

SEQ ID NO: 209 - protein, 112 aa, Artificial
  Synthetic construct
DIVMTQTPLSLSVTPGQPASISCRSSQSLVHSRGKTYLHWYLQKPGQSPQLLIYKVSNRFSGVPDRFSGSGSGTDFTLKISRVEAEDVGVYYCSQSTHYPFTFGQGTKLEIK

SEQ ID NO: 210 - protein, 112 aa, Artificial
  Synthetic construct
DIVMTQTPLSLSVTPGQPASISCRSSQSLVHLRGNTYLHWYLQKPGQSPQLLIYKVSNRFSGVPDRFSGSGSGTDFTLKISRVEAEDVGVYYCSQSTHYPFTFGQGTKLEIK

SEQ ID NO: 211 - protein, 112 aa, Artificial
  Synthetic construct
DIVMTQTPLSLSVTPGQPASISCRSSQSLVHSRGNTYLHWYLQKPGQSPQLLIYIVSNRFSGVPDRFSGSGSGTDFTLKISRVEAEDVGVYYCSQSTHYPFTFGQGTKLEIK

SEQ ID NO: 212 - protein, 112 aa, Artificial; identical to SEQ ID NO: 179
  Synthetic construct

SEQ ID NO: 213 - protein, 112 aa, Artificial; identical to SEQ ID NO: 179
  Synthetic construct

SEQ ID NO: 214 - protein, 112 aa, Artificial; identical to SEQ ID NO: 191
  Synthetic construct

SEQ ID NO: 215 - protein, 112 aa, Artificial; identical to SEQ ID NO: 196
  Synthetic construct

SEQ ID NO: 216 - protein, 112 aa, Artificial; identical to SEQ ID NO: 195
  Synthetic construct

SEQ ID NO: 217 - protein, 112 aa, Artificial
  Synthetic construct
DIVMTQTPLSLSVTPGQPASISCRSSQSLRHSRGNTYLHWYLQKPGQSPQLLIYKVSNRFHGVPDRFSGSGSGTDFTLKISRVEAEDVGVYYCSQSTHYPFTFGQGTKLEIK

SEQ ID NO: 218 - protein, 112 aa, Artificial
  Synthetic construct
DIVMTQTPLSLSVTPGQPASISCRSSKSLVHSRGNTYLHWYLQKPGQSPQLLIYKVANRFSGVPDRFSGSGSGTDFTLKISRVEAEDVGVYYCSQSTHYPFTFGQGTKLEIK

SEQ ID NO: 219 - protein, 112 aa, Artificial
  Synthetic construct
DIVMTQTPLSLSVTPGQPASISCRSSKSLVHSRGNTFLHWYLQKPGQSPQLLIYKVSVRFSGVPDRFSGSGSGTDFTLKISRVEAEDVGVYYCSQSTHYPFTFGQGTKLEIK

SEQ ID NO: 220 - protein, 112 aa, Artificial
  Synthetic construct
DIVMTQTPLSLSVTPGQPASISCRSSQSLVHSRGNTYLHWYLQKPGQSPQLLIYKVSNNFSGVPDRFSGSGSGTDFTLKISRVEAEDVGVYYCSQSTHYPFTFGQGTKLEIK

SEQ ID NO: 221 - protein, 112 aa, Artificial
  Synthetic construct
DIVMTQTPLSLSVTPGQPASISCRSSQSLVHSRGNTFLHWYLQKPGQSPQLLIYKVDNRFSGVPDRFSGSGSGTDFTLKISRVEAEDVGVYYCSQSTHYPFTFGQGTKLEIK

SEQ ID NO: 222 - protein, 112 aa, Artificial
  Synthetic construct
DIVMTQTPLSLSVTPGQPASISCRSSRSLVHSRGNTFLHWYLQKPGQSPQLLIYKVTNRFSGVPDRFSGSGSGTDFTLKISRVEAEDVGVYYCSQSTHYPFTFGQGTKLEIK

SEQ ID NO: 223 - protein, 112 aa, Artificial
  Synthetic construct
DIVMTQTPLSLSVTPGQPASISCRSSQSLRHSRGNTYLHWYLQKPGQSPQLLIYKVSNIFSGVPDRFSGSGSGTDFTLKISRVEAEDVGVYYCSQSTHYPFTFGQGTKLEIK

SEQ ID NO: 224 - protein, 112 aa, Artificial
  Synthetic construct
DIVMTQTPLSLSVTPGQPASISCRSSKSLVHSRGNTFLHWYLQKPGQSPQLLIYKVSTRFSGVPDRFSGSGSGTDFTLKISRVEAEDVGVYYCSQSTHYPFTFGQGTKLEIK

SEQ ID NO: 225 - protein, 112 aa, Artificial; identical to SEQ ID NO: 196
  Synthetic construct

SEQ ID NO: 226 - protein, 112 aa, Artificial
  Synthetic construct
DIVMTQTPLSLSVTPGQPASISCRSSQSLVHSRGNTFLHWYLQKPGQSPQLLIYKVRNRFSGVPDRFSGSGSGTDFTLKISRVEAEDVGVYYCSQSTHYPFTFGQGTKLEIK

SEQ ID NO: 227 - protein, 112 aa, Artificial
  Synthetic construct
DIVMTQTPLSLSVTPGQPASISCRSSQSLRHSRGNTYLHWYLQKPGQSPQLLIYKVPNRFSGVPDRFSGSGSGTDFTLKISRVEAEDVGVYYCSQSTHYPFTFGQGTKLEIK

SEQ ID NO: 228 - protein, 112 aa, Artificial
  Synthetic construct
DIVMTQTPLSLSVTPGQPASISCRSSQSLVHSRGNTFLHWYLQKPGQSPQLLIYKVSNRFVGVPDRFSGSGSGTDFTLKISRVEAEDVGVYYCSQSTHYPFTFGQGTKLEIK

SEQ ID NO: 229 - protein, 112 aa, Artificial
  Synthetic construct
DIVMTQTPLSLSVTPGQPASISCRSSQSLRHSRGNTYLHWYLQKPGQSPQLLIYKVSNRISGVPDRFSGSGSGTDFTLKISRVEAEDVGVYYCSQSTHYPFTFGQGTKLEIK

SEQ ID NO: 230 - protein, 112 aa, Artificial
  Synthetic construct
DIVMTQTPLSLSVTPGQPASISCRSSRSLVHSRGNTYLHWYLQKPGQSPQLLIYKVSNRFTGVPDRFSGSGSGTDFTLKISRVEAEDVGVYYCSQSTHYPFTFGQGTKLEIK

SEQ ID NO: 231 - protein, 112 aa, Artificial
  Synthetic construct
DIVMTQTPLSLSVTPGQPASISCRSSQSLRHSRGNTYLHWYLQKPGQSPQLLIYKVSNRNSGVPDRFSGSGSGTDFTLKISRVEAEDVGVYYCSQSTHYPFTFGQGTKLEIK

SEQ ID NO: 232 - protein, 112 aa, Artificial
  Synthetic construct
DIVMTQTPLSLSVTPGQPASISCRSSKSLVHSRGNTYLHWYLQKPGQSPQLLIYKVHNRFSGVPDRFSGSGSGTDFTLKISRVEAEDVGVYYCSQSTHYPFTFGQGTKLEIK

SEQ ID NO: 233 - protein, 112 aa, Artificial
  Synthetic construct
DIVMTQTPLSLSVTPGQPASISCRSSQSLKHSRGNTYLHWYLQKPGQSPQLLIYKVSTRFSGVPDRFSGSGSGTDFTLKISRVEAEDVGVYYCSQSTHYPFTFGQGTKLEIK

SEQ ID NO: 234 - protein, 112 aa, Artificial
  Synthetic construct
DIVMTQTPLSLSVTPGQPASISCRSSQSLVHSRGNTFLHWYLQKPGQSPQLLIYKVSNRFIGVPDRFSGSGSGTDFTLKISRVEAEDVGVYYCSQSTHYPFTFGQGTKLEIK

SEQ ID NO: 235 - protein, 112 aa, Artificial
  Synthetic construct
DIVMTQTPLSLSVTPGQPASISCRSSQSLKHSHGNTYLHWYLQKPGQSPQLLIYKVSNRFIGVPDRFSGSGSGTDFTLKISRVEAEDVGVYYCSQSTHYPFTFGQGTKLEIK

SEQ ID NO: 236 - protein, 112 aa, Artificial
  Synthetic construct
DIVMTQTPLSLSVTPGQPASISCRSSKSLVHSRGNTYLHWYLQKPGQSPQLLIYKVSNRFIGVPDRFSGSGSGTDFTLKISRVEAEDVGVYYCSQSTHYPFTFGQGTKLEIK

SEQ ID NO: 237 - protein, 112 aa, Artificial
  Synthetic construct
DIVMTQTPLSLSVTPGQPASISCRSSQSLVHSRGNTYLHWYLQKPGQSPQLLIYKVSNRFIGVPDRFSGSGSGTDFTLKISRVEAEDVGVYYCSQSTHYPFTFGQGTKLEIK

SEQ ID NO: 238 - protein, 112 aa, Artificial; identical to SEQ ID NO: 237
  Synthetic construct

SEQ ID NO: 239 - protein, 112 aa, Artificial
  Synthetic construct
DIVMTQTPLSLSVTPGQPASISCRSSQSLKHSRGNTFLHWYLQKPGQSPQLLIYKVSNRFIGVPDRFSGSGSGTDFTLKISRVEAEDVGVYYCSQSTHYPFTFGQGTKLEIK

SEQ ID NO: 240 - protein, 112 aa, Artificial
  Synthetic construct
DIVMTQTPLSLSVTPGQPASISCRSSRSLVHSRGNTYLHWYLQKPGQSPQLLIYKVSNRFIGVPDRFSGSGSGTDFTLKISRVEAEDVGVYYCSQSTHYPFTFGQGTKLEIK

SEQ ID NO: 241 - protein, 112 aa, Artificial
  Synthetic construct
DIVMTQTPLSLSVTPGQPASISCRSSRSLVHSRGNTYLHWYLQKPGQSPQLLIYKVSNRFIGVPDRFSGSGSGTDFTLKISRVEAEDVGVYYCSQSTHLPFTFGQGTKLEIK

SEQ ID NO: 242 - protein, 112 aa, Artificial
  Synthetic construct
DIVMTQTPLSLSVTPGQPASISCRSSQSLKHSRGNTYLHWYLQKPGQSPQLLIYKVSNRFIGVPDRFSGSGSGTDFTLKISRVEAEDVGVYYCSQSTHYPFTFGQGTKLEIK

SEQ ID NO: 243 - protein, 112 aa, Artificial; identical to SEQ ID NO: 242
  Synthetic construct

SEQ ID NO: 244 - protein, 10 aa, Artificial
  Synthetic construct
  MISC_FEATURE (1)..(1): X is G or H
  MISC_FEATURE (3)..(3): X is S, H, or P
  MISC_FEATURE (5)..(5): X is T, G, R, N, or P
  MISC_FEATURE (6)..(6): X is D or  W
  MISC_FEATURE (7)..(7): X is Y or F
  MISC_FEATURE (8)..(8): X is N or H
  MISC_FEATURE (9)..(9): X is M, I, L or T
  MISC_FEATURE (10)..(10): X is N, S, G, or H
XYXFXXXXXX

SEQ ID NO: 245 - protein, 17 aa, Artificial
  Synthetic construct
  MISC_FEATURE (5)..(5): X is N, M, A or E
VINPXYGTTDYNQRFKG

SEQ ID NO: 246 - protein, 10 aa, Artificial
  Synthetic construct
  MISC_FEATURE (3)..(3): X is  Y, A or P
  MISC_FEATURE (4)..(4): X is  A, S, F, L. H, Y or W
  MISC_FEATURE (5)..(5): X is  T or P
  MISC_FEATURE (6)..(6): X is G or S
  MISC_FEATURE (9)..(9): X is P, A, V, G, L or T
YDXXXXTGXY

SEQ ID NO: 247 - protein, 16 aa, Artificial
  Synthetic construct
  MISC_FEATURE (1)..(1): X is R or V
  MISC_FEATURE (3)..(3): X is S or H
  MISC_FEATURE (4)..(4): X is Q, K, A or R
  MISC_FEATURE (6)..(6): X is L or V
  MISC_FEATURE (7)..(7): X is V, K or R
  MISC_FEATURE (9)..(9): X is S, N, A, R or L
  MISC_FEATURE (10)..(10): X is R, H, N or Y
  MISC_FEATURE (12)..(12): X is N, R or K
  MISC_FEATURE (13)..(13): X is T or V
  MISC_FEATURE (14)..(14): X is Y, F or W
  MISC_FEATURE (15)..(15): X is L, T, S, H or F
XSXXSXXHXXGXXXXH

SEQ ID NO: 248 - protein, 7 aa, Artificial
  Synthetic construct
  MISC_FEATURE (1)..(1): X is K or I
  MISC_FEATURE (3)..(3): X is T, D, S, A, R, P or H
  MISC_FEATURE (4)..(4): X is N, V or T
  MISC_FEATURE (5)..(5): X is R, N or I
  MISC_FEATURE (6)..(6): X is F, N or I
  MISC_FEATURE (7)..(7): X is S, H, V, T or I
XVXXXXX

SEQ ID NO: 249 - protein, 9 aa, Artificial
  Synthetic construct
  MISC_FEATURE (1)..(1): X is S or N
  MISC_FEATURE (3)..(3): X is S or T
  MISC_FEATURE (4)..(4): X is T, M or L
  MISC_FEATURE (5)..(5): X is H or S
  MISC_FEATURE (6)..(6): X is L, Y, I,  V or E
XQXXXXPFT

SEQ ID NO: 250 - DNA, 468 bp, Homo sapiens
atgactcctgggaagacctcattggtgtcactgctactgctgctgagcctggaggccatagtgaaggcaggaatcacaatcccacgaaatccaggatgcccaaattctgaggacaagaacttcccccggactgtgatggtcaacctgaacatccataaccggaataccaataccaatcccaaaaggtcctcagattactacaaccgatccacctcaccttggaatctccaccgcaatgaggaccctgagagatatccctctgtgatctgggaggcaaagtgccgccacttgggctgcatcaacgctgatgggaacgtggactaccacatgaactctgtccccatccagcaagagatcctggtcctgcgcagggagcctccacactgccccaactccttccggctggagaagatactggtgtccgtgggctgcacctgtgtcaccccgattgtccaccatgtggcctaa

SEQ ID NO: 251 - DNA, 462 bp, Oryctolagus cuniculus
atgtcgcttgggaggatttcatctgtgtcactgctgctgctgctgtgtttggtggctactgtgaagaatggaatagcaatgccgcgaaatccaggatgtccaaatgctgaggacaagaacttcccccagaatgtaaaagtcagcctgaacatccttaacaagagtgtaaattcccgaaggccttcagactactacaatcgatctacttcaccttggactctccaccgcaacgaggatcgtgagagatatccctctgtgatctgggaggccaagtgccgccacttgggctgtgtcaatgctgaagggaatgaggaccaccacatgaactctgtcccaatccagcaagagatcctggtcctacgcagggagtcccagcactgcccacactcattccggctggagaagatgctggtggctgtaggatgcacctgtgtaacccccatcatccatcacatggcctaa

SEQ ID NO: 252 - DNA, 477 bp, Rattus rattus
atgagtccccggagaattccatccatgtgcctgatgctgttgctgctactgaacctggaggctacagtgaaggcagcggtactcatccctcaaagttcagtgtgtccaaacgccgaggccaataactttctccagaacgtgaaggtcaacctgaaagtcctcaactcccttagctcaaaagcgagctccagaaggccctcagactacctcaaccgttccacttcaccctggactctgagccgcaatgaggaccctgatagatatccttctgtgatctgggaggcacagtgccgccaccagcgctgtgtcaacgctgaggggaagttggaccaccacatgaattctgttctcatccagcaagagatcctggtcctgaagagggagcctgagaagtgccccttcactttccgggtggagaagatgctggtgggcgtgggctgcacctgcgtttcctctattgtccgccatgcgtcctaa

SEQ ID NO: 253 - DNA, 468 bp, Macaca fascicularis
atgactcctgggaagacctcattggtgctactgctgctgctgctgagcctggaggccatagtgaaggcaggaatagcaatcccacgaaattcaggatgcccaaattctgaggacaagaacttcccccggactgtgatggtcaacctgaacatccataaccggaataccagtaccaatcccaaaaggtcctcagattactacaaccgatccacctcaccttggaatctccaccgcaatgaggaccctgagagatatccctctgtgatctgggaggcaaaatgccgccacttaggctgcgtcaaggctgatgggaacgtagactaccacatgaactctgtccccatccagcaagagatcctggtcctgcgcagggagcctcggcactgccccaactccttccggctggagaagatactggtgtccgtgggctgcacctgtgtcacccccattgtccaccatgtagcctaa

SEQ ID NO: 254 - DNA, 477 bp, Mus sp.
atgagtccagggagagcttcatctgtgtctctgatgctgttgctgctgctgagcctggcggctacagtgaaggcagcagcgatcatccctcaaagctcagcgtgtccaaacactgaggccaaggacttcctccagaatgtgaaggtcaacctcaaagtctttaactcccttggcgcaaaagtgagctccagaaggccctcagactacctcaaccgttccacgtcaccctggactctccaccgcaatgaagaccctgatagatatccctctgtgatctgggaagctcagtgccgccaccagcgctgtgtcaatgcggagggaaagctggaccaccacatgaattctgttctcatccagcaagagatcctggtcctgaagagggagcctgagagctgccccttcactttcagggtcgagaagatgctggtgggtgtgggctgcacctgcgtggcctcgattgtccgccaggcagcctaa

SEQ ID NO: 255 - protein, 107 aa, Homo sapiens [sequence omitted]

SEQ ID NO: 256 - protein, 105 aa, Homo sapiens
QPKAAPSVTLFPPSSEELQANKATLVCLISDFYPGAVTVAWKADSSPVKAGVETTTPSKQSNNKYAASSYLSLTPEQWKSHRSYSCQVTHEGSTVEKTVAPTECS

SEQ ID NO: 257 - protein, 330 aa, Homo sapiens
ASFKGPSVFPLAPSSKSTSGGTAALGCLVKDYFPEPVTVSWNSGALTSGVHTFPAVLQSSGLYSLSSVVTVPSSSLGTQTYICNVNHKPSNTKVDKKVEPKSCDKTHTCPPCPAPELLGGPSVFLFPPKPKDTLMISRTPEVTCVVVDVSHEDPEVKFNWYVDGVEVHNAKTKPREEQYNSTYRVVSVLTVLHQDWLNGKEYKCKVSNKALPAPIEKTISKAKGQPREPQVYTLPPSREEMTKNQVSLTCLVKGFYPSDIAVEWESNGQPENNYKTTPPVLEWETWRRLYWKLTVDKSRWQQGNVFSCSVMHEALHNHYTQKSLSLSPGK

SEQ ID NO: 258 - protein, 325 aa, Homo sapiens
ASTKGPSVFPLAPCSRSTSESTAALGCLVKDYFPEPVTVSWNSGALTSGVHTFPAVLQSSGLYSLSSVVTVPSSNFGTQTYTCNVDHKPSNTKVDKTVERKCCVECPPCPAPPVAGPSVFLFPPKPKDTLMISRTPEVTCVVVDVSHEDPEVQFNWYDGVEVHNAKTKPREEQFNSTFRVVSVLTVVHQDWLNGKEYKCKVSNKGLPAPIEKTISKTKGQPREPQVYTLPPSREEMTKNQVSLTCLVKGFYPSDIAVEWESNGQPENNYKTTPPMLDSDGSFFLYSKLTVDKSRWQQGNVFSCSVMHEALHNHYTQKSLSLSPGK

SEQ ID NO: 259 - protein, 377 aa, Homo sapiens
ASTKGPSVFPLAPCSRSTSGGTAALGCLVKDYFPEPVTVSWNSGALTSGVHTFPAVLQSSGLYSLSSVVTVPSSSLGTQTYTCNVNHKPSNTKVDKRVELKTPLGDTTHTCPRCPEPKSCDTPPPCPRCPEPKSCDTPPPCPRCPEPKSCDTPPPCPRCPAPELLGGPSVFLFPPKPKDTLMISRTPEVTCVVVDVSHEDPEVQFKWYVDGVEVHNAKTKPREEQYNSTFRVVSVLTVLHQDWLNGKEYKCKVSNKALPAPIEKTISKTKGQPREPQVYTLPPSREEMTKNQVSLTCLVKGFYPSDIAVEWESSGQPENNYNTTPPMLDSDGSFFLYSKLTVDKSRWQQGNIFSCSVMHEALHNRFTQKSLSLSPGK

SEQ ID NO: 260 - protein, 326 aa, Homo sapiens
ASTKGPSVFPLAPCSRSTSESTAALGCLVKDYFPEPVTVSWNSGALTSGVHTFPAVLQSSGLYSLSSVVTVPSSSLGTKTYTCNVDHKPSNTKVDKRVESKYGPPCPPCPAPEFLGGPSVFLFPPKPKDTLMISRTPEVTCVVVDVSQEDPEVQFNWYVDGVEVHNAKTKPREEQFNSTYRVVSVLTVLHQDWLNGKEYKCKVSNKGLPSSIEKTISKAKGQPREPQVYTLPPSQEEMTKNQVSLTCLVKGFYPSDIAVEWESNGQPENNYKTTPPVLDSDGSFFLYSRLTVDKSRWQEGNVFSCSVMHEALHNHYTQKSLSLSLG

SEQ ID NO: 261 - protein, 10 aa, Artificial
  Synthetic construct
YDAFTGTGAY

SEQ ID NO: 262 - protein, 25 aa, Artificial [sequence omitted]

SEQ ID NO: 263 - protein, 14 aa, Artificial
  Synthetic construct
WVRQAPGQGLEWMG

SEQ ID NO: 264 - protein, 32 aa, Artificial
  Synthetic construct
RVTITADESTSTAYMELSSLRSEDTAVYYCAR

SEQ ID NO: 265 - protein, 11 aa, Artificial
  Synthetic construct
WGQGTLVTVSS

SEQ ID NO: 266 - protein, 23 aa, Artificial
  Synthetic construct
DIVMTQTPLSLSVTPGQPASISC

SEQ ID NO: 267 - protein, 15 aa, Artificial
  Synthetic construct
WYLQKPGQSPQLLIY

SEQ ID NO: 268 - protein, 32 aa, Artificial
  Synthetic construct
GVPDRFSGSGSGTDFTLKISRVEAEDVGVYYC

SEQ ID NO: 269 - protein, 10 aa, Artificial
  Synthetic construct
FGQGTKLEIK

SEQ ID NO: 270 - protein, 119 aa, Mus sp.
QVQLQQSRPELVKPGASVKISCKASGYSFTDYNMNWVKQSNGKSLEWIGVINPNYGTTDYNQRFKGKATLTVDQSSRTAYMQLNSLTSEDSAVYYCVIYDYATGTGGYWGQGSPLTVSS

SEQ ID NO: 271 - protein, 112 aa, Mus sp.
DVVLTQTPLSLPVSLGDQASISCRSSQSLVHSNGNTYLHWYLQKPGQSPKLLIYKVSNRFSGVPDRFSGSGSGTDFTLKISRVEAEDLGVYFCSQSTHVPFTFGSGTKLEIK

SEQ ID NO: 272 - protein, 107 aa, Homo sapiens [sequence omitted]

SEQ ID NO: 273 - protein, 445 aa, Homo sapiens
QVQLVQSGAEVKKPGSSVKVSCKASGYSFTDYHIHWVRQAPGQGLEWMGVINPMYGTTDYNQRFKGRVTITADESTSTAYMELSSLRSEDTAVYYCARYDYFTGTGVYWGQGTLVTVSSASTKGPSVFPLAPCSRSTSESTAALGCLVKDYFPEPVTVSWNSGALTSGVHTFPAVLQSSGLYSLSSVVTVPSSSLGTKTYTCNVDHKPSNTKVDKRVESKYGPPCPPCPAPEFLGGPSVFLFPPKPKDTLMISRTPEVTCVVVDVSQEDPEVQFNWYVDGVEVHNAKTKPREEQFNSTYRVVSVLTVLHQDWLNGKEYKCKVSNKGLPSSIEKTISKAKGQPREPQVYTLPPSQEEMTKNQVSLTCLVKGFYPSDIAVEWESNGQPENNYKTTPPVLDSDGSFFLYSRLTVDKSRWQEGNVFSCSVMHEALHNHYTQKSLSLSLG

SEQ ID NO: 274 - protein, 219 aa, Homo sapiens
DIVMTQTPLSLSVTPGQPASISCRSSRSLVHSRGNTYLHWYLQKPGQSPQLLIYKVSNRFIGVPDRFSGSGSGTDFTLKISRVEAEDVGVYYCSQSTHLPFTFGQGTKLEIKRTVAAPSVFIFPPSDEQLKSGTASVVCLLNNFYPREAKVQWKVDNALQSGNSQESVTEQDSKDSTYSLSSTLTLSKADYEKHKVYACEVTHQGLSSPVTKSFNRGEC

SEQ ID NO: 275 - protein, 10 aa, Homo sapiens
ADGNVDYHMN

SEQ ID NO: 276 - protein, 7 aa, Homo sapiens
DGNVDYH

SEQ ID NO: 277 - protein, 107 aa, Artificial [sequence omitted]

SEQ ID NO: 278 - protein, 326 aa, Artificial; identical to SEQ ID NO: 260
  Synthetic construct

SEQ ID NO: 279 - protein, 219 aa, Artificial; identical to SEQ ID NO: 274
  Synthetic construct

SEQ ID NO: 280 - protein, 445 aa, Artificial; identical to SEQ ID NO: 273
  Synthetic construct